European Patent Application EP 4 467 636 A1, published November 27, 2024. Title: BACILLUS VELEZENSIS AND USE THEREOF. Applicant: Moon (Guangzhou) Biotech Co., Ltd. Application WO PCT/CN2023/073307, filed January 20, 2023. The sequence listing filed with the application follows.

SEQUENCE LISTING (4 sequences)

SEQ ID NO: 1 - DNA, 1388 bp, synthetic construct
  misc_feature 1..1388: note = Reference sequence 1
  source 1..1388: mol_type = other DNA
tcgtagacgagcataatccgtagcttgctccctgatgttagcggcggacgggtgagtaacacgtgggtaacctgcctgtaagactgggataactccgggaaaccggggctaataccggatggttgtttgaaccgcatggttcagacataaaaggtggcttcggctaccacttacagatggacccgcggcgcattagctagttggtgaggtaacggctcaccaaggcaacgatgcgtagccgacctgagagggtgatcggccacactgggactgagacacggcccagactcctacgggaggcagcagtagggaatcttccgcaatggacgaaagtctgacggagcaacgccgcgtgagtgatgaaggttttcggatcgtaaagctctgttgttagggaagaacaagtgccgttcaaatagggcggcaccttgacggtacctaaccagaaagccacggctaactacgtgccagcagccgcggtaatacgtaggtggcaagcgttgtccggaattattgggcgtaaagggctcgcaggcggtttcttaagtctgatgtgaaagcccccggctcaaccggggagggtcattggaaactggggaacttgagtgcagaagaggagagtggaattccacgtgtagcggtgaaatgcgtagagatgtggaggaacaccagtggcgaaggcgactctctggtctgtaactgacgctgaggagcgaaagcgtggggagcgaacaggattagataccctggtagtccacgccgtaaacgatgagtgctaagtgttagggggtttccgccccttagtgctgcagctaacgcattaagcactccgcctggggagtacggtcgcaagactgaaactcaaaggaattgacgggggcccgcacaagcggtggagcatgtggtttaattcgaagcaacgcgaagaaccttaccaggtcttgacatcctctgacaatcctagagataggacgtccccttcgggggcagagtgacaggtggtgcatggttgtcgtcagctcgtgtcgtgagatgttgggttaagtcccgcaacgagcgcaacccttgatcttagttgccagcattcagttgggcactctaaggtgactgccggtgacaaaccggaggaaggtggggatgacgtcaaatcatcatgccccttatgacctgggctacacacgtgctacaatggacagaacaaagggcagcgaaaccgcgaggttaagccaatcccacaaatctgttctcagttcggatcgcagtctgcaactcgactgcgtgaagctggaatcgctagtaatcgcggatcagcatgccgcggtgaatacgttcccgggccttgtacacaccgcccgtctacaccacgagagtttgtaacacccgaagtc

SEQ ID NO: 2 - DNA, 1407 bp, synthetic construct
  misc_feature 1..1407: note = Reference sequence 2
  source 1..1407: mol_type = other DNA
agtcgagcggacagaagggagcttgctcccggatgttagcggcggacgggtgagtaacacgtgggtaacctgcctgtaagactgggataactccgggaaaccggagctaataccggatagttccttgaaccgcatggttcaaggatgaaagacggtttcggctgtcacttacagatggacccgcggcgcattagctagttggtggggtaatggctcaccaaggcgacgatgcgtagccgacctgagagggtgatcggccacactgggactgagacacggcccagactcctacgggaggcagcagtagggaatcttccgcaatggacgaaagtctgacggagcaacgccgcgtgagtgatgaaggttttcggatcgtaaagctctgttgttagggaagaacaagtgcgagagtaactgctcgcaccttgacggtacctaaccagaaagccacggctaactacgtgccagcagccgcggtaatacgtaggtggcaagcgttgtccggaattattgggcgtaaagggctcgcaggcggtttcttaagtctgatgtgaaagcccccggctcaaccggggagggtcattggaaactgggaaacttgagtgcagaagaggagagtggaattccacgtgtagcggtgaaatgcgtagagatgtggaggaacaccagtggcgaaggcgactctctggtctgtaactgacgctgaggagcgaaagcgtggggagcgaacaggattagataccctggtagtccacgccgtaaacgatgagtgctaagtgttagggggtttccgccccttagtgctgcagctaacgcattaagcactccgcctggggagtacggtcgcaagactgaaactcaaaggaattgacgggggcccgcacaagcggtggagcatgtggtttaattcgaagcaacgcgaagaaccttaccaggtcttgacatcctctgacaaccctagagatagggctttcccttcggggacagagtgacaggtggtgcatggttgtcgtcagctcgtgtcgtgagatgttgggttaagtcccgcaacgagcgcaacccttgatcttagttgccagcatttagttgggcactctaaggtgactgccggtgacaaaccggaggaaggtggggatgacgtcaaatcatcatgccccttatgacctgggctacacacgtgctacaatggacagaacaaagggctgcgagaccgcaaggtttagccaatcccataaatctgttctcagttcggatcgcagtctgcaactcgactgcgtgaagctggaatcgctagtaatcgcggatcagcatgccgcggtgaatacgttcccgggccttgtacacaccgcccgtcacaccacgagagtttgcaacacccgaagtcggtgaggtaacctttatggagcc

SEQ ID NO: 3 - DNA, 20 bp, synthetic construct
  misc_feature 1..20: note = Primer 27F
  source 1..20: mol_type = other DNA
agagtttgatcctggctcag

SEQ ID NO: 4 - DNA, 19 bp, synthetic construct
  misc_feature 1..19: note = Primer 1492R
  source 1..19: mol_type = other DNA
ggttaccttgttacgactt